European Patent Application EP 4 234 722 A2, published August 30, 2023. Title: DETECTING COLORECTAL NEOPLASM. Applicant: MAYO FOUNDATION FOR MEDICAL EDUCATION AND RESEARCH. Application EP. The sequence listing filed with the application follows.

SEQUENCE LISTING (110 sequences)

SEQ ID NO: 1 - DNA, 21 bp, synthetic construct
  misc_feature 1..21: note = Synthetic
  source 1..21: mol_type = other DNA
gggagtgagggtagggcgttc

SEQ ID NO: 2 - DNA, 25 bp, synthetic construct
  misc_feature 1..25: note = Synthetic
  source 1..25: mol_type = other DNA
ctcgcaaccccttcgaattaacccg

SEQ ID NO: 3 - DNA, 25 bp, synthetic construct
  misc_feature 1..25: note = Synthetic
  source 1..25: mol_type = other DNA
tgcgtaggtgatagggaggggttac

SEQ ID NO: 4 - DNA, 25 bp, synthetic construct
  misc_feature 1..25: note = Synthetic
  source 1..25: mol_type = other DNA
acaaaacacatcctattaacgcgaa

SEQ ID NO: 5 - DNA, 19 bp, synthetic construct
  misc_feature 1..19: note = Synthetic
  source 1..19: mol_type = other DNA
gagtcgcggtttcgttttc

SEQ ID NO: 6 - DNA, 19 bp, synthetic construct
  misc_feature 1..19: note = Synthetic
  source 1..19: mol_type = other DNA
gacgcgacgaccgaaaaac

SEQ ID NO: 7 - DNA, 23 bp, synthetic construct
  misc_feature 1..23: note = Synthetic
  source 1..23: mol_type = other DNA
tgcacaccccgaggcggtcccgg

SEQ ID NO: 8 - DNA, 23 bp, synthetic construct
  misc_feature 1..23: note = Synthetic
  source 1..23: mol_type = other DNA
cgcccccaaaataaaaaaacgaa

SEQ ID NO: 9 - skipped

SEQ ID NO: 10 - DNA, 20 bp, synthetic construct
  misc_feature 1..20: note = Synthetic
  source 1..20: mol_type = other DNA
gcgtttaggttggtcggaga

SEQ ID NO: 11 - DNA, 20 bp, synthetic construct
  misc_feature 1..20: note = Synthetic
  source 1..20: mol_type = other DNA
cctaaccaacgcactcaacc

SEQ ID NO: 12 - DNA, 21 bp, synthetic construct
  misc_feature 1..21: note = Synthetic
  source 1..21: mol_type = other DNA
cgtagcgtggcgttttagcgc

SEQ ID NO: 13 - DNA, 26 bp, synthetic construct
  misc_feature 1..26: note = Synthetic
  source 1..26: mol_type = other DNA
tcgaaaaccccgacgaaacgaaaacg

SEQ ID NO: 14 - DNA, 25 bp, synthetic construct
  misc_feature 1..25: note = Synthetic
  source 1..25: mol_type = other DNA
gcgtaaggtcgaatatttgagtcga

SEQ ID NO: 15 - DNA, 25 bp, synthetic construct
  misc_feature 1..25: note = Synthetic
  source 1..25: mol_type = other DNA
aaaatactacccaccaaccaccgaa

SEQ ID NO: 16 - DNA, 19 bp, synthetic construct
  misc_feature 1..19: note = Synthetic
  source 1..19: mol_type = other DNA
gtcgtcgttcgagagggta

SEQ ID NO: 17 - DNA, 22 bp, synthetic construct
  misc_feature 1..22: note = Synthetic
  source 1..22: mol_type = other DNA
cgaacaaaaacgaacgaacgaa

SEQ ID NO: 18 - DNA, 33 bp, synthetic construct
  misc_feature 1..33: note = Synthetic
  source 1..33: mol_type = other DNA
tcgattttatttttgttgtcgttgtagattcgc

SEQ ID NO: 19 - DNA, 33 bp, synthetic construct
  misc_feature 1..33: note = Synthetic
  source 1..33: mol_type = other DNA
gaaaaaactaaaaaacgacaaaaaaacccgacg

SEQ ID NO: 20 - DNA, 28 bp, synthetic construct
  misc_feature 1..28: note = Synthetic
  source 1..28: mol_type = other DNA
ggaacgagtgatagtcggatagttcgtc

SEQ ID NO: 21 - DNA, 18 bp, synthetic construct
  misc_feature 1..18: note = Synthetic
  source 1..18: mol_type = other DNA
cgcccgaaaacgaccccg

SEQ ID NO: 22 - DNA, 31 bp, synthetic construct
  misc_feature 1..31: note = Synthetic
  source 1..31: mol_type = other DNA
cggggatgattttatgtagtcggagtttcgc

SEQ ID NO: 23 - DNA, 24 bp, synthetic construct
  misc_feature 1..24: note = Synthetic
  source 1..24: mol_type = other DNA
cccgccgaatactcgatcaactcg

SEQ ID NO: 24 - DNA, 34 bp, synthetic construct
  misc_feature 1..34: note = Synthetic
  source 1..34: mol_type = other DNA
gcgaataaataaacgttaatttgttgtttgtttc

SEQ ID NO: 25 - DNA, 25 bp, synthetic construct
  misc_feature 1..25: note = Synthetic
  source 1..25: mol_type = other DNA
ccgaacgcgtataaataccgcactt

SEQ ID NO: 26 - DNA, 28 bp, synthetic construct
  misc_feature 1..28: note = Synthetic
  source 1..28: mol_type = other DNA
cggttttatttattatgattcgtagcgg

SEQ ID NO: 27 - DNA, 24 bp, synthetic construct
  misc_feature 1..24: note = Synthetic
  source 1..24: mol_type = other DNA
cgactaccctaaacaacgcatcgc

SEQ ID NO: 28 - DNA, 23 bp, synthetic construct
  misc_feature 1..23: note = Synthetic
  source 1..23: mol_type = other DNA
cgagttcggtagttgtacgtaga

SEQ ID NO: 29 - DNA, 27 bp, synthetic construct
  misc_feature 1..27: note = Synthetic
  source 1..27: mol_type = other DNA
cgaaatacgaacgcgaaatctaaaact

SEQ ID NO: 30 - DNA, 19 bp, synthetic construct
  misc_feature 1..19: note = Synthetic
  source 1..19: mol_type = other DNA
gcgacgtagtcgtcgttgt

SEQ ID NO: 31 - DNA, 19 bp, synthetic construct
  misc_feature 1..19: note = Synthetic
  source 1..19: mol_type = other DNA
ccaacgcgaaaaaaacgcg

SEQ ID NO: 32 - DNA, 19 bp, synthetic construct
  misc_feature 1..19: note = Synthetic
  source 1..19: mol_type = other DNA
gaggcggacgtcgcggtac

SEQ ID NO: 33 - DNA, 25 bp, synthetic construct
  misc_feature 1..25: note = Synthetic
  source 1..25: mol_type = other DNA
cgccacgacgcgaatcttaactacg

SEQ ID NO: 34 - DNA, 22 bp, synthetic construct
  misc_feature 1..22: note = Synthetic
  source 1..22: mol_type = other DNA
ggatcgagggagtaggagtcgc

SEQ ID NO: 35 - DNA, 22 bp, synthetic construct
  misc_feature 1..22: note = Synthetic
  source 1..22: mol_type = other DNA
cgaaaccgaacctaacgcgacg

SEQ ID NO: 36 - DNA, 24 bp, synthetic construct
  misc_feature 1..24: note = Synthetic
  source 1..24: mol_type = other DNA
agttttttcgcgcgttttttttgc

SEQ ID NO: 37 - DNA, 21 bp, synthetic construct
  misc_feature 1..21: note = Synthetic
  source 1..21: mol_type = other DNA
gccgaatctccgccttacacg

SEQ ID NO: 38 - DNA, 23 bp, synthetic construct
  misc_feature 1..23: note = Synthetic
  source 1..23: mol_type = other DNA
gtttaattttcggtttcgtcgtc

SEQ ID NO: 39 - DNA, 20 bp, synthetic construct
  misc_feature 1..20: note = Synthetic
  source 1..20: mol_type = other DNA
cgccgaggcggttttttgcg

SEQ ID NO: 40 - DNA, 18 bp, synthetic construct
  misc_feature 1..18: note = Synthetic
  source 1..18: mol_type = other DNA
cgctacgaaacactccga

SEQ ID NO: 41 - DNA, 21 bp, synthetic construct
  misc_feature 1..21: note = Synthetic
  source 1..21: mol_type = other DNA
cggttttcgttcgttttttcg

SEQ ID NO: 42 - DNA, 21 bp, synthetic construct
  misc_feature 1..21: note = Synthetic
  source 1..21: mol_type = other DNA
ccacggacggttcgtttatcg

SEQ ID NO: 43 - DNA, 18 bp, synthetic construct
  misc_feature 1..18: note = Synthetic
  source 1..18: mol_type = other DNA
ccgccttctacgcgacta

SEQ ID NO: 44 - DNA, 34 bp, synthetic construct; identical to SEQ ID NO: 24
  misc_feature 1..34: note = Synthetic
  source 1..34: mol_type = other DNA

SEQ ID NO: 45 - DNA, 21 bp, synthetic construct
  misc_feature 1..21: note = Synthetic
  source 1..21: mol_type = other DNA
ccacggacgcgcacttcctta

SEQ ID NO: 46 - DNA, 25 bp, synthetic construct
  misc_feature 1..25: note = Synthetic
  source 1..25: mol_type = other DNA
ccgaacgcgtataaataccgcactt

SEQ ID NO: 47 - DNA, 23 bp, synthetic construct
  misc_feature 1..23: note = Synthetic
  source 1..23: mol_type = other DNA
cgagttcggtagttgtacgtaga

SEQ ID NO: 48 - DNA, 20 bp, synthetic construct
  misc_feature 1..20: note = Synthetic
  source 1..20: mol_type = other DNA
cgccgaggtcgtcgataccg

SEQ ID NO: 49 - DNA, 27 bp, synthetic construct
  misc_feature 1..27: note = Synthetic
  source 1..27: mol_type = other DNA
cgaaatacgaacgcgaaatctaaaact

SEQ ID NO: 50 - DNA, 19 bp, synthetic construct
  misc_feature 1..19: note = Synthetic
  source 1..19: mol_type = other DNA
gcgacgtagtcgtcgttgt

SEQ ID NO: 51 - DNA, 21 bp, synthetic construct
  misc_feature 1..21: note = Synthetic
  source 1..21: mol_type = other DNA
ccacggacggaaaacgcgaaa

SEQ ID NO: 52 - DNA, 19 bp, synthetic construct
  misc_feature 1..19: note = Synthetic
  source 1..19: mol_type = other DNA
ccaacgcgaaaaaaacgcg

SEQ ID NO: 53 - skipped

SEQ ID NO: 54 - DNA, 19 bp, synthetic construct
  misc_feature 1..19: note = Synthetic
  source 1..19: mol_type = other DNA
tcggagtcgagtttagcgc

SEQ ID NO: 55 - DNA, 21 bp, synthetic construct
  misc_feature 1..21: note = Synthetic
  source 1..21: mol_type = other DNA
ccacggacgcggcgttcgcga

SEQ ID NO: 56 - DNA, 24 bp, synthetic construct
  misc_feature 1..24: note = Synthetic
  source 1..24: mol_type = other DNA
cgaaatcgaaaaaacaaaaaccgc

SEQ ID NO: 57 - DNA, 23 bp, synthetic construct
  misc_feature 1..23: note = Synthetic
  source 1..23: mol_type = other DNA
cgagttcggtagttgtacgtaga

SEQ ID NO: 58 - DNA, 20 bp, synthetic construct
  misc_feature 1..20: note = Synthetic
  source 1..20: mol_type = other DNA
cgccgaggtcgtcgataccg

SEQ ID NO: 59 - DNA, 20 bp, synthetic construct
  misc_feature 1..20: note = Synthetic
  source 1..20: mol_type = other DNA
cgccgaggtcgtcgataccg

SEQ ID NO: 60 - DNA, 19 bp, synthetic construct
  misc_feature 1..19: note = Synthetic
  source 1..19: mol_type = other DNA
gtcgtcgttcgagagggta

SEQ ID NO: 61 - DNA, 21 bp, synthetic construct
  misc_feature 1..21: note = Synthetic
  source 1..21: mol_type = other DNA
ccacggacgatcggtttcgtt

SEQ ID NO: 62 - DNA, 22 bp, synthetic construct
  misc_feature 1..22: note = Synthetic
  source 1..22: mol_type = other DNA
cgaacaaaaacgaacgaacgaa

SEQ ID NO: 63 - DNA, 20 bp, synthetic construct
  misc_feature 1..20: note = Synthetic
  source 1..20: mol_type = other DNA
gcgtttaggttggtcggaga

SEQ ID NO: 64 - DNA, 20 bp, synthetic construct
  misc_feature 1..20: note = Synthetic
  source 1..20: mol_type = other DNA
cgccgaggctacgaaccgaa

SEQ ID NO: 65 - DNA, 20 bp, synthetic construct
  misc_feature 1..20: note = Synthetic
  source 1..20: mol_type = other DNA
cctaaccaacgcactcaacc

SEQ ID NO: 66 - DNA, 21 bp, synthetic construct
  misc_feature 1..21: note = Synthetic
  source 1..21: mol_type = other DNA
ttagcgacgtagtcgtcgttg

SEQ ID NO: 67 - DNA, 21 bp, synthetic construct
  misc_feature 1..21: note = Synthetic
  source 1..21: mol_type = other DNA
ccacggacgcgaaaacgcgaa

SEQ ID NO: 68 - DNA, 19 bp, synthetic construct
  misc_feature 1..19: note = Synthetic
  source 1..19: mol_type = other DNA
cccaacgcgaaaaaaacgc

SEQ ID NO: 69 - DNA, 21 bp, synthetic construct
  misc_feature 1..21: note = Synthetic
  source 1..21: mol_type = other DNA
gtatagcgcgatttcgtagcg

SEQ ID NO: 70 - DNA, 20 bp, synthetic construct
  misc_feature 1..20: note = Synthetic
  source 1..20: mol_type = other DNA
cgccgaggcgaacatcctcc

SEQ ID NO: 71 - DNA, 21 bp, synthetic construct
  misc_feature 1..21: note = Synthetic
  source 1..21: mol_type = other DNA
aattacctacgctatccgccc

SEQ ID NO: 72 - DNA, 22 bp, synthetic construct
  misc_feature 1..22: note = Synthetic
  source 1..22: mol_type = other DNA
cgtcgcgtttttcggttatacg

SEQ ID NO: 73 - DNA, 21 bp, synthetic construct
  misc_feature 1..21: note = Synthetic
  source 1..21: mol_type = other DNA
ccacggacggcaccgtaaaac

SEQ ID NO: 74 - DNA, 21 bp, synthetic construct
  misc_feature 1..21: note = Synthetic
  source 1..21: mol_type = other DNA
cgcgaaaactaaaaaaccgcg

SEQ ID NO: 75 - DNA, 27 bp, synthetic construct
  misc_feature 1..27: note = Synthetic
  source 1..27: mol_type = other DNA
aaacgttaatttgttgtttgtttcgtt

SEQ ID NO: 76 - DNA, 24 bp, synthetic construct
  misc_feature 1..24: note = Synthetic
  source 1..24: mol_type = other DNA
actttccgaacgcgtataaatacc

SEQ ID NO: 77 - DNA, 35 bp, synthetic construct
  misc_feature 1..35: note = Synthetic
  source 1..35: mol_type = other DNA
gcgaataaataaacgttaatttgttgtttgtttcg

SEQ ID NO: 78 - DNA, 23 bp, synthetic construct
  misc_feature 1..23: note = Synthetic
  source 1..23: mol_type = other DNA
gttgcgaggttaggttgtaatcg

SEQ ID NO: 79 - DNA, 20 bp, synthetic construct
  misc_feature 1..20: note = Synthetic
  source 1..20: mol_type = other DNA
cgccgaggcgtccatttaac

SEQ ID NO: 80 - DNA, 22 bp, synthetic construct
  misc_feature 1..22: note = Synthetic
  source 1..22: mol_type = other DNA
cgccgcttaccttaataatccc

SEQ ID NO: 81 - DNA, 19 bp, synthetic construct
  misc_feature 1..19: note = Synthetic
  source 1..19: mol_type = other DNA
gagtcgcggtttcgttttc

SEQ ID NO: 82 - DNA, 20 bp, synthetic construct
  misc_feature 1..20: note = Synthetic
  source 1..20: mol_type = other DNA
cgccgaggcgcgttcgtttt

SEQ ID NO: 83 - DNA, 19 bp, synthetic construct
  misc_feature 1..19: note = Synthetic
  source 1..19: mol_type = other DNA
gacgcgacgaccgaaaaac

SEQ ID NO: 84 - DNA, 21 bp, synthetic construct
  misc_feature 1..21: note = Synthetic
  source 1..21: mol_type = other DNA
cggttttcgttcgttttttcg

SEQ ID NO: 85 - DNA, 21 bp, synthetic construct
  misc_feature 1..21: note = Synthetic
  source 1..21: mol_type = other DNA
ccacggacggttcgtttatcg

SEQ ID NO: 86 - DNA, 18 bp, synthetic construct
  misc_feature 1..18: note = Synthetic
  source 1..18: mol_type = other DNA
ccgccttctacgcgacta

SEQ ID NO: 87 - DNA, 23 bp, synthetic construct
  misc_feature 1..23: note = Synthetic
  source 1..23: mol_type = other DNA
gtttaattttcggtttcgtcgtc

SEQ ID NO: 88 - DNA, 20 bp, synthetic construct
  misc_feature 1..20: note = Synthetic
  source 1..20: mol_type = other DNA
cgccgaggcggttttttgcg

SEQ ID NO: 89 - DNA, 18 bp, synthetic construct
  misc_feature 1..18: note = Synthetic
  source 1..18: mol_type = other DNA
cgctacgaaacactccga

SEQ ID NO: 90 - DNA, 19 bp, synthetic construct
  misc_feature 1..19: note = Synthetic
  source 1..19: mol_type = other DNA
gcgtttaggttggtcggag

SEQ ID NO: 91 - DNA, 20 bp, synthetic construct
  misc_feature 1..20: note = Synthetic
  source 1..20: mol_type = other DNA
cgccgaggccgaaaaactac

SEQ ID NO: 92 - DNA, 19 bp, synthetic construct
  misc_feature 1..19: note = Synthetic
  source 1..19: mol_type = other DNA
acgcactcaacctacgaac

SEQ ID NO: 93 - DNA, 19 bp, synthetic construct
  misc_feature 1..19: note = Synthetic
  source 1..19: mol_type = other DNA
gcgacgtagtcgtcgttgt

SEQ ID NO: 94 - DNA, 21 bp, synthetic construct
  misc_feature 1..21: note = Synthetic
  source 1..21: mol_type = other DNA
ccacggacggaaaacgcgaaa

SEQ ID NO: 95 - DNA, 19 bp, synthetic construct
  misc_feature 1..19: note = Synthetic
  source 1..19: mol_type = other DNA
ccaacgcgaaaaaaacgcg

SEQ ID NO: 96 - DNA, 35 bp, synthetic construct; identical to SEQ ID NO: 77
  misc_feature 1..35: note = Synthetic
  source 1..35: mol_type = other DNA

SEQ ID NO: 97 - DNA, 21 bp, synthetic construct
  misc_feature 1..21: note = Synthetic
  source 1..21: mol_type = other DNA
ccacggacgcgcacttcctta

SEQ ID NO: 98 - DNA, 24 bp, synthetic construct
  misc_feature 1..24: note = Synthetic
  source 1..24: mol_type = other DNA
actttccgaacgcgtataaatacc

SEQ ID NO: 99 - DNA, 36 bp, synthetic construct
  misc_feature 1..36: note = Synthetic
  source 1..36: mol_type = other DNA
gatcgagggagcaggagccgcggctgacgggtcgcg

SEQ ID NO: 100 - DNA, 35 bp, synthetic construct
  misc_feature 1..35: note = Synthetic
  source 1..35: mol_type = other DNA
cggtgccgagagctgccagagagttggattctgcg

SEQ ID NO: 101 - DNA, 24 bp, synthetic construct
  misc_feature 1..24: note = Synthetic
  source 1..24: mol_type = other DNA
gcgagcgggcaagggcgggcgagc

SEQ ID NO: 102 - DNA, 28 bp, synthetic construct
  misc_feature 1..28: note = Synthetic
  source 1..28: mol_type = other DNA
acctgcgggccgaagggctgctctccgg

SEQ ID NO: 103 - DNA, 29 bp, synthetic construct
  misc_feature 1..29: note = Synthetic
  source 1..29: mol_type = other DNA
aggagacgcgggagcgcggggtaggtagc

SEQ ID NO: 104 - DNA, 34 bp, synthetic construct
  misc_feature 1..34: note = Synthetic
  source 1..34: mol_type = other DNA
ggcatcctcccggtgatggaagcagccgccgccg

SEQ ID NO: 105 - DNA, 34 bp, synthetic construct
  misc_feature 1..34: note = Synthetic
  source 1..34: mol_type = other DNA
ggaaggcgcggcgctcggtcagcactgacagcag

SEQ ID NO: 106 - DNA, 39 bp, synthetic construct
  misc_feature 1..39: note = Synthetic
  source 1..39: mol_type = other DNA
tcgccgagctctccccaaacttcctgcatgctgaacttt

SEQ ID NO: 107 - DNA, 31 bp, synthetic construct
  misc_feature 1..31: note = Synthetic
  source 1..31: mol_type = other DNA
ccgtccatttggccaagtctgcagccgagcc

SEQ ID NO: 108 - DNA, 33 bp, synthetic construct
  misc_feature 1..33: note = Synthetic
  source 1..33: mol_type = other DNA
ctgcgtccgtccgtcggccgggcagtctgtcca

SEQ ID NO: 109 - DNA, 48 bp, synthetic construct
  misc_feature 1..48: note = Synthetic
  source 1..48: mol_type = other DNA
tccctcgcgcgtggcttccgccttctgcgcggctggggtgcccggtgg

SEQ ID NO: 110 - DNA, 26 bp, synthetic construct
  misc_feature 1..26: note = Synthetic
  source 1..26: mol_type = other DNA
gcgggacactccgaaggcgcaaggag